European Patent Application EP 4 484 555 A1, published January 1, 2025. Title: An agent for enhancing productivity of a virus vector and a method for producing a virus vector. Applicant: Nippon Medical School Foundation. The sequence listing filed with the application follows.

SEQUENCE LISTING (8 sequences)

SEQ ID NO: 1 - DNA, 20 bp, synthetic construct
  misc_feature 1..20: note = Synthetic DNA
  source 1..20: mol_type = other DNA
tgacttccggctttctaagg

SEQ ID NO: 2 - DNA, 18 bp, synthetic construct
  misc_feature 1..18: note = Synthetic DNA
  source 1..18: mol_type = other DNA
tgtggcaggaagccaaac

SEQ ID NO: 3 - DNA, 20 bp, synthetic construct
  misc_feature 1..20: note = Synthetic DNA
  source 1..20: mol_type = other DNA
ggagccttggagttctttgc

SEQ ID NO: 4 - DNA, 20 bp, synthetic construct
  misc_feature 1..20: note = Synthetic DNA
  source 1..20: mol_type = other DNA
cctctggctgggattatgct

SEQ ID NO: 5 - DNA, 20 bp, synthetic construct
  misc_feature 1..20: note = Synthetic DNA
  source 1..20: mol_type = other DNA
gcggcggaaaatagcctttg

SEQ ID NO: 6 - DNA, 21 bp, synthetic construct
  misc_feature 1..21: note = Synthetic DNA
  source 1..21: mol_type = other DNA
gatcacacgttccacctcatc

SEQ ID NO: 7 - DNA, 19 bp, synthetic construct
  misc_feature 1..19: note = Synthetic DNA
  source 1..19: mol_type = other DNA
gctttgctatgagctgctg

SEQ ID NO: 8 - DNA, 20 bp, synthetic construct
  misc_feature 1..20: note = Synthetic DNA
  source 1..20: mol_type = other DNA
gcctgagcagtttggagatg